European Patent Specification EP 3 632 903 B1, published October 11, 2023. Title: COMPOUND USED AS AUTOPHAGY REGULATOR, AND PREPARATION METHOD THEREFOR AND USES THEREOF. Applicant: WIGEN BIOMEDICINE TECHNOLOGY (SHANGHAI) CO., LTD. The sequence listing filed with the application follows.

SEQUENCE LISTING (2 sequences)

SEQ ID NO: 1 - protein, 356 aa, Artificial Sequence
  GST-LC3B
MSPILGYWKIKGLVQPTRLLLEYLEEKYEEHLYERDEGDKWRNKKFELGLEFPNLPYYIDGDVKLTQSMAIIRYIADKHNMLGGCPKERAEISMLEGAVLDIRYGVSRIAYSKDFETLKVDFLSKLPEMLKMFEDRLCHKTYLNGDHVTHPDFMLYDALDVVLYMDPMCLDAFPKLVCFKKRIEAIPQIDKYLKSSKYIAWPLQGWQATFGGGDHPPKSDLEVLFQGPLGSMPSEKTFKQRRTFEQRVEDVRLIREQHPTKIPVIIERYKGEKQLPVLDKTKFLVPDHVNMSELIKIIRRRLQLNANQAFFLLVNGHSMVSVSTPISEVYESEKDEDGFLYMVYASQETFGMKLSV

SEQ ID NO: 2 - protein, 15 aa, Artificial Sequence
  N-terminal FITC-labeled peptide
GGDDDWTHLSSKEVD